European Patent Specification EP 3 621 635 B1, published September 2, 2026. Title: Enveloped Virus Resistant to Complement Inactivation for the Treatment of Cancer. Applicant: Wellstat ImmunoTherapeutics Corporation. The sequence listing filed with the application follows.

SEQUENCE LISTING (3 sequences)

SEQ ID NO: 1 - DNA, 6606 bp, Artificial Sequence
  Mammalian cell expression construct.
  misc_feature (1064)..(1165): Code for secretory signal peptide
  misc_feature (1166)..(2119): Code for SCR of CD55
  misc_feature (2120)..(2164): Code for (G4S1)3 linker
  misc_feature (2165)..(2227): Code for CD8 transmembrane domain
  misc_feature (2228)..(2260): Code for truncated CD8 intracellular domain
tcaatattggccattagccatattattcattggttatatagcataaatcaatattggctattggccattgcatacgttgtatctatatcataatatgtacatttatattggctcatgtccaatatgaccgccatgttggcattgattattgactagttattaatagtaatcaattacggggtcattagttcatagcccatatatggagttccgcgttacataacttacggtaaatggcccgcctggctgaccgcccaacgacccccgcccattgacgtcaataatgacgtatgttcccatagtaacgccaatagggactttccattgacgtcaatgggtggagtatttacggtaaactgcccacttggcagtacatcaagtgtatcatatgccaagtccgccccctattgacgtcaatgacggtaaatggcccgcctggcattatgcccagtacatgaccttacgggactttcctacttggcagtacatctacgtattagtcatcgctattaccatggtgatgcggttttggcagtacaccaatgggcgtggatagcggtttgactcacggggatttccaagtctccaccccattgacgtcaatgggagtttgttttggcaccaaaatcaacgggactttccaaaatgtcgtaataaccccgccccgttgacgcaaatgggcggtaggcgtgtacggtgggaggtctatataagcagagctcgtttagtgaaccgtcagatcactagaagctttattgcggtagtttatcacagttaaattgctaacgcagtcagtgcttctgacacaacagtctcgaacttaagctgcagaagttggtcgtgaggcactgggcaggtaagtatcaaggttacaagacaggtttaaggagaccaatagaaactgggcttgtcgagacagagaagactcttgcgtttctgataggcacctattggtcttactgacatccactttgcctttctctccacaggtgtccactcccagttcaattacagctcttaaggctagagtacttaatacgactcactataggctagcgccaccatgacagtggccagaccttctgtgcctgccgccctgcctctgctgggagaactgcctagactgctgctgctggtgctgctgtgtctgcctgccgtgtggggcgattgtggcctgcctcccgatgtgcctaatgcccagcctgccctggaaggcagaaccagcttccccgaggacaccgtgatcacctacaagtgcgaggaatccttcgtgaagatccccggcgagaaggatagcgtgatctgcctgaagggcagccagtggagcgacatcgaagagttctgcaacagatcctgcgaggtgcccacccggctgaatagcgcctctctgaagcagccctacatcacccagaactacttccctgtgggcaccgtggtggaatacgagtgcagacccggctacagaagagagccctccctgagccctaagctgacctgcctgcagaacctgaagtggtccaccgccgtggagttctgtaaaaagaagtcctgccccaaccctggcgagatccggaacggccagattgatgtgcctggcggcatcctgttcggcgccacaatcagcttcagctgcaacaccggctacaagctgttcggcagcacctccagcttttgcctgatcagcggcagcagcgtgcagtggagtgaccctctgcctgagtgcagagagatctactgccctgccccccctcagatcgacaacggcatcattcagggcgagcgggaccactacggctacaggcagagcgtgacctacgcctgcaacaagggcttcaccatgatcggcgagcacagcatctactgcaccgtgaacaacgacgagggcgagtggagcggcccaccccctgagtgtagaggcaagagcctgaccagcaaggtgccccccaccgtgcagaaacccaccaccgtgaatgtgcctaccaccgaggtgtccccaaccagccagaaaacaaccaccaagaccaccacccccaacgcccaggccaccagatctacccctgtgtccaggaccaccaagcacttccacgagacaacccctaacaagggcagcggcacaaccggtggcggaggatctggcggcggaggaagcggagggggaggatccatctatatctgggcccctctggccggcacctgtggcgtgctgctgctgtctctcgtgatcaccctgtactgcaaccaccggaaccggcggagagtgtgatgagaattcacgcgtggtacctctagagtcgaccctctagggcggccaattccgcccctctccctcccccccccctaacgttactggccgaagccgcttggaataaggccggtgtgcgtttgtctatatgttattttccaccatattgccgtcttttggcaatgtgagggcccggaaacctggccctgtcttcttgacgagcattcctaggggtctttcccctctcgccaaaggaatgcaaggtctgttgaatgtcgtgaaggaagcagttcctctggaagcttcttgaagacaaacaacgtctgtagcgaccctttgcaggcagcggaaccccccacctggcgacaggtgcctctgcggccaaaagccacgtgtataagatacacctgcaaaggcggcacaaccccagtgccacgttgtgagttggatagttgtggaaagagtcaaatggctctcctcaagcgtattcaacaaggggctgaaggatgcccagaaggtaccccattgtatgggatctgatctggggcctcggtgcacatgctttacatgtgtttagtcgaggttaaaaaaacgtctaggccccccgaaccacggggacgtggttttcctttgaaaaacacgatgataagcttgccacaacccgggataattcctgcagccaatatgggatcggccattgaacaagatggattgcacgcaggttctccggccgcttgggtggagaggctattcggctatgactgggcacaacagacaatcggctgctctgatgccgccgtgttccggctgtcagcgcaggggcgcccggttctttttgtcaagaccgacctgtccggtgccctgaatgaactgcaggacgaggcagcgcggctatcgtggctggccacgacgggcgttccttgcgcagctgtgctcgacgttgtcactgaagcgggaagggactggctgctattgggcgaagtgccggggcaggatctcctgtcatctcaccttgctcctgccgagaaagtatccatcatggctgatgcaatgcggcggctgcatacgcttgatccggctacctgcccattcgaccaccaagcgaaacatcgcatcgagcgagcacgtactcggatggaagccggtcttgtcgatcaggatgatctggacgaagagcatcaggggctcgcgccagccgaactgttcgccaggctcaaggcgcgcatgcccgacggcgatgatctcgtcgtgacccatggcgatgcctgcttgccgaatatcatggtggaaaatggccgcttttctggattcatcgactgtggccggctgggtgtggcggaccgctatcaggacatagcgttggctacccgtgatattgctgaagagcttggcggcgaatgggctgaccgcttcctcgtgctttacggtatcgccgctcccgattcgcagcgcatcgccttctatcgccttcttgacgagttcttctgaggggatcaattctgggcggcctcgagaataaacaatcattattttcattggatctgtgtgttggttttttgtgtgggcttgggggagggggaggccagaatgactccaagagctacaggaaggcaggtcagagaccccactggacaaacagtggctggactctgcaccataacacacaatcaacaggggagtgagctggatcgagctgctcgagatccgggctggcgtaatagcgaagaggcccgcaccgatcgcccttcccaacagttgcgcagcctgaatggcgaatggacgcgccctgtagcggcgcattaagcgcggcgggtgtggtggttacgcgcagcgtgaccgctacacttgccagcgccctagcgcccgctcctttcgctttcttcccttcctttctcgccacgttcgccggctttccccgtcaagctctaaatcgggggctccctttagggttccgatttagtgctttacggcacctcgaccccaaaaaacttgattagggtgatggttcacgtagtgggccatcgccctgatagacggtttttcgccctttgacgttggagtccacgttctttaatagtggactcttgttccaaactggaacaacactcaaccctatctcggtctattcttttgatttataagggattttgccgatttcggcctattggttaaaaaatgagctgatttaacaaaaatttaacgcgaattttaacaaaatattaacgcttacaatttcctgatgcggtattttctccttacgcatctgtgcggtatttcacaccgcatatggtgcactctcagtacaatctgctctgatgccgcatagttaagccagccccgacacccgccaacacccgctgacgcgccctgacgggcttgtctgctcccggcatccgcttacagacaagctgtgaccgtctccgggagctgcatgtgtcagaggttttcaccgtcatcaccgaaacgcgcgagacgaaagggcctcgtgatacgcctatttttataggttaatgtcatgataataatggtttcttagacgtcaggtggcacttttcggggaaatgtgcgcggaacccctatttgtttatttttctaaatacattcaaatatgtatccgctcatgagacaataaccctgataaatgcttcaataatattgaaaaaggaagagtatgagtattcaacatttccgtgtcgcccttattcccttttttgcggcattttgccttcctgtttttgctcacccagaaacgctggtgaaagtaaaagatgctgaagatcagttgggtgcacgagtgggttacatcgaactggatctcaacagcggtaagatccttgagagttttcgccccgaagaacgttttccaatgatgagcacttttaaagttctgctatgtggcgcggtattatcccgtattgacgccgggcaagagcaactcggtcgccgcatacactattctcagaatgacttggttgagtactcaccagtcacagaaaagcatcttacggatggcatgacagtaagagaattatgcagtgctgccataaccatgagtgataacactgcggccaacttacttctgacaacgatcggaggaccgaaggagctaaccgcttttttgcacaacatgggggatcatgtaactcgccttgatcgttgggaaccggagctgaatgaagccataccaaacgacgagcgtgacaccacgatgcctgtagcaatggcaacaacgttgcgcaaactattaactggcgaactacttactctagcttcccggcaacaattaatagactggatggaggcggataaagttgcaggaccacttctgcgctcggcccttccggctggctggtttattgctgataaatctggagccggtgagcgtgggtctcgcggtatcattgcagcactggggccagatggtaagccctcccgtatcgtagttatctacacgacggggagtcaggcaactatggatgaacgaaatagacagatcgctgagataggtgcctcactgattaagcattggtaactgtcagaccaagtttactcatatatactttagattgatttaaaacttcatttttaatttaaaaggatctaggtgaagatcctttttgataatctcatgaccaaaatcccttaacgtgagttttcgttccactgagcgtcagaccccgtagaaaagatcaaaggatcttcttgagatcctttttttctgcgcgtaatctgctgcttgcaaacaaaaaaaccaccgctaccagcggtggtttgtttgccggatcaagagctaccaactctttttccgaaggtaactggcttcagcagagcgcagataccaaatactgttcttctagtgtagccgtagttaggccaccacttcaagaactctgtagcaccgcctacatacctcgctctgctaatcctgttaccagtggctgctgccagtggcgataagtcgtgtcttaccgggttggactcaagacgatagttaccggataaggcgcagcggtcgggctgaacggggggttcgtgcacacagcccagcttggagcgaacgacctacaccgaactgagatacctacagcgtgagctatgagaaagcgccacgcttcccgaagggagaaaggcggacaggtatccggtaagcggcagggtcggaacaggagagcgcacgagggagcttccagggggaaacgcctggtatctttatagtcctgtcgggtttcgccacctctgacttgagcgtcgatttttgtgatgctcgtcaggggggcggagcctatggaaaaacgccagcaacgcggcctttttacggttcctggccttttgctggccttttgctcacatggctcgacagatct

SEQ ID NO: 2 - protein, 399 aa, Artificial Sequence
  Fusion protein
  SIGNAL (1)..(34): Secretory signal peptide
  PEPTIDE (35)..(352): SCR of CD55
  MISC_FEATURE (353)..(367): (G4S1)3 linker
  TRANSMEM (368)..(388): CD8 transmembrane domain
  DOMAIN (389)..(399): Truncated CD8 intracellular domain
MTVARPSVPAALPLLGELPRLLLLVLLCLPAVWGDCGLPPDVPNAQPALEGRTSFPEDTVITYKCEESFVKIPGEKDSVICLKGSQWSDIEEFCNRSCEVPTRLNSASLKQPYITQNYFPVGTVVEYECRPGYRREPSLSPKLTCLQNLKWSTAVEFCKKKSCPNPGEIRNGQIDVPGGILFGATISFSCNTGYKLFGSTSSFCLISGSSVQWSDPLPECREIYCPAPPQIDNGIIQGERDHYGYRQSVTYACNKGFTMIGEHSIYCTVNNDEGEWSGPPPECRGKSLTSKVPPTVQKPTTVNVPTTEVSPTSQKTTTKTTTPNAQATRSTPVSRTTKHFHETTPNKGSGTTGGGGSGGGGSGGGGSIYIWAPLAGTCGVLLLSLVITLYCNHRNRRRV

SEQ ID NO: 3 - protein, 365 aa, Artificial Sequence
  Mature fusion protein (after cleavage of signal peptide).
  PEPTIDE (1)..(318): SCR of CD55
  MISC_FEATURE (319)..(333): (G4S1)3 linker
  TRANSMEM (334)..(354): CD8 transmembrane domain
  DOMAIN (355)..(365): Trunated CD8 intracellular domain
DCGLPPDVPNAQPALEGRTSFPEDTVITYKCEESFVKIPGEKDSVICLKGSQWSDIEEFCNRSCEVPTRLNSASLKQPYITQNYFPVGTVVEYECRPGYRREPSLSPKLTCLQNLKWSTAVEFCKKKSCPNPGEIRNGQIDVPGGILFGATISFSCNTGYKLFGSTSSFCLISGSSVQWSDPLPECREIYCPAPPQIDNGIIQGERDHYGYRQSVTYACNKGFTMIGEHSIYCTVNNDEGEWSGPPPECRGKSLTSKVPPTVQKPTTVNVPTTEVSPTSQKTTTKTTTPNAQATRSTPVSRTTKHFHETTPNKGSGTTGGGGSGGGGSGGGGSIYIWAPLAGTCGVLLLSLVITLYCNHRNRRRV